European Patent Specification EP 4 405 376 B1, published August 27, 2025. Title: Method for the fermentative production of L-lysine using C. glutamicum strains expressing modified gluconate repressor proteins GntR1 and GntR2. Applicant: Evonik Operations GmbH. Application EP. The sequence listing filed with the application follows.

SEQUENCE LISTING (11 sequences)

SEQ ID NO: 1 - DNA, 753 bp, Corynebacterium glutamicum ATCC 13032
  misc_feature 1..753: note = nucleotide sequence comprising locus_tag NCgl2440 disclosed inGenbank NC_003450
  source 1..753: mol_type = genomic DNA
atgaccccagcaaacgaaagtcctatgactaatccattaggttctgcccccaccccagccaagccacttcttgacagtgttcttgatgagctcggtcaagatatcatcagtggcaaggttgctgtcggagataccttcaagctgatggacatcggcgagcgttttggcatttcccgcacagtggcacgcgaagcgatgcgcgctttggagcagctcggtcttgtcgcttcttcacgtcgcattggcattactgttttgccacaggaagagtgggctgtttttgataagtccatcattcgctggcgtctcaatgacgaaggtcagcgtgaaggccagcttcagtctcttaccgagcttcgtattgctattgaaccgattgccgcgcgcagcgttgctcttcacgcgtcaaccgccgagctcgagaaaatccgcgcgctcgcaacagagatgcgtcagttgggtgaatctggtcagggtgcgtcccagcgcttcctcgaagcggacgtcactttccacgagctcatcttgcgttattgccacaatgagatgttcgctgcactgattccgtcgattagcgcggttcttgtcggccgcaccgagctcggcctgcagcctgatctgccggcgcacgaggcgctagacaaccacgataagcttgccgacgccctccttaaccgcgacgccgacgccgcagaaactgcgtcccgaaacatcctcaatgaggtgcgcagcgcgctgggcacgctgaactaa

SEQ ID NO: 2 - DNA, 741 bp, Corynebacterium glutamicum ATCC 13032
  misc_feature 1..741: note = nucleotide sequence comprising locus_tag NCgl1650 disclosed in
  source 1..741: mol_type = genomic DNA
atgtccgcagctttacctcacacagcagcagatcccgtacacaccaccccagcgaaaccgctgctcgatcatgtcttagattcactaggacgcagcatcatcagtggtgaaatggaagccggtagcacattcaaactgcaagacatcggtgaaaaattcggtatctcccgcaccgtcgccagagaagccatgcgtgccttagagcaacttgggttggtggcctcatcgagacgaattggtattacagtgctctcgcacgagcactgggctgtctttgacaaagccattattcgctggcgcctcgaagatgagcgtcaacgtgaacagcaactgcagtcactcaccgaacttcgtattgccattgaaccaattgctgcacgcagtgttgcccttcatgcatcgagcgcagagattgctatcatcggtgatcttgctgcacgaatgcgtaacctcggtgaagctggtcgtggcgcatcacaagaattcctagacgcagatgtgaaatttcatgagcttattttgcagtattgccataatgagatgttcgctgccatggcaccacccataaaagctgtactagtcgggcgcaccacacttggccttcaacccgatcgacctgccgaagaagtcttggacaatcatgatgctctcgcacacgcactaagtgttcgtaatgcagacctcgccgaaaaagcatccaggagcattctgaatgaggtgcgcgacgcactgacctcgtaa

SEQ ID NO: 3 - DNA, 1266 bp, Corynebacterium glutamicum ATCC 13032
  misc_feature 1..1266: note = /note="lysC_T311I"/note="exchange of nucleobase cytosine (c) at position 932 togive thymine (t). The acc codon for threonine is altered to atccodon for isoleucine"
  source 1..1266: mol_type = genomic DNA
gtggccctggtcgtacagaaatatggcggttcctcgcttgagagtgcggaacgcattagaaacgtcgctgaacggatcgttgccaccaagaaggctggaaatgatgtcgtggttgtctgctccgcaatgggagacaccacggatgaacttctagaacttgcagcggcagtgaatcccgttccgccagctcgtgaaatggatatgctcctgactgctggtgagcgtatttctaacgctctcgtcgccatggctattgagtcccttggcgcagaagcccaatctttcacgggctctcaggctggtgtgctcaccaccgagcgccacggaaacgcacgcattgttgatgtcactccaggtcgtgtgcgtgaagcactcgatgagggcaagatctgcattgttgctggtttccagggtgttaataaagaaacccgcgatgtcaccacgttgggtcgtggtggttctgacaccactgcagttgcgttggcagctgctttgaacgctgatgtgtgtgagatttactcggacgttgacggtgtgtataccgctgacccgcgcatcgttcctaatgcacagaagctggaaaagctcagcttcgaagaaatgctggaacttgctgctgttggctccaagattttggtgctgcgcagtgttgaatacgctcgtgcattcaatgtgccacttcgcgtacgctcgtcttatagtaatgatcccggcactttgattgccggctctatggaggatattcctgtggaagaagcagtccttaccggtgtcgcaaccgacaagtccgaagccaaagtaaccgttctgggtatttccgataagccaggcgaggctgcgaaggttttccgtgcgttggctgatgcagaaatcaacattgacatggttctgcagaacgtctcttctgtagaagacggcaccaccgacatcatcttcacctgccctcgttccgacggccgccgcgcgatggagatcttgaagaagcttcaggttcagggcaactggaccaatgtgctttacgacgaccaggtcggcaaagtctccctcgtgggtgctggcatgaagtctcacccaggtgttaccgcagagttcatggaagctctgcgcgatgtcaacgtgaacatcgaattgatttccacctctgagattcgtatttccgtgctgatccgtgaagatgatctggatgctgctgcacgtgcattgcatgagcagttccagctgggcggcgaagacgaagccgtcgtttatgcaggcaccggacgctaa

SEQ ID NO: 4 - DNA, 753 bp, Corynebacterium glutamicum ATCC 13032
  misc_feature 1..753: note = gntR1_R102E
  source 1..753: mol_type = genomic DNA
atgaccccagcaaacgaaagtcctatgactaatccattaggttctgcccccaccccagccaagccacttcttgacagtgttcttgatgagctcggtcaagatatcatcagtggcaaggttgctgtcggagataccttcaagctgatggacatcggcgagcgttttggcatttcccgcacagtggcacgcgaagcgatgcgcgctttggagcagctcggtcttgtcgcttcttcacgtcgcattggcattactgttttgccacaggaagagtgggctgtttttgataagtccatcattcgctgggaactcaatgacgaaggtcagcgtgaaggccagcttcagtctcttaccgagcttcgtattgctattgaaccgattgccgcgcgcagcgttgctcttcacgcgtcaaccgccgagctcgagaaaatccgcgcgctcgcaacagagatgcgtcagttgggtgaatctggtcagggtgcgtcccagcgcttcctcgaagcggacgtcactttccacgagctcatcttgcgttattgccacaatgagatgttcgctgcactgattccgtcgattagcgcggttcttgtcggccgcaccgagctcggcctgcagcctgatctgccggcgcacgaggcgctagacaaccacgataagcttgccgacgccctccttaaccgcgacgccgacgccgcagaaactgcgtcccgaaacatcctcaatgaggtgcgcagcgcgctgggcacgctgaactaa

SEQ ID NO: 5 - protein, 250 aa, Corynebacterium glutamicum ATCC 13032
  REGION 1..250: note = gluconate repressor protein variant GntR1_R102E wherein the aminoacid Arg in position 102 of the wildtype sequence is replaced bythe amino acid Glu
MTPANESPMTNPLGSAPTPAKPLLDSVLDELGQDIISGKVAVGDTFKLMDIGERFGISRTVAREAMRALEQLGLVASSRRIGITVLPQEEWAVFDKSIIRWELNDEGQREGQLQSLTELRIAIEPIAARSVALHASTAELEKIRALATEMRQLGESGQGASQRFLEADVTFHELILRYCHNEMFAALIPSISAVLVGRTELGLQPDLPAHEALDNHDKLADALLNRDADAAETASRNILNEVRSALGTLN

SEQ ID NO: 6 - DNA, 753 bp, Corynebacterium glutamicum ATCC 13032
  misc_feature 1..753: note = gntR1_R102C
  source 1..753: mol_type = genomic DNA
atgaccccagcaaacgaaagtcctatgactaatccattaggttctgcccccaccccagccaagccacttcttgacagtgttcttgatgagctcggtcaagatatcatcagtggcaaggttgctgtcggagataccttcaagctgatggacatcggcgagcgttttggcatttcccgcacagtggcacgcgaagcgatgcgcgctttggagcagctcggtcttgtcgcttcttcacgtcgcattggcattactgttttgccacaggaagagtgggctgtttttgataagtccatcattcgctggtgtctcaatgacgaaggtcagcgtgaaggccagcttcagtctcttaccgagcttcgtattgctattgaaccgattgccgcgcgcagcgttgctcttcacgcgtcaaccgccgagctcgagaaaatccgcgcgctcgcaacagagatgcgtcagttgggtgaatctggtcagggtgcgtcccagcgcttcctcgaagcggacgtcactttccacgagctcatcttgcgttattgccacaatgagatgttcgctgcactgattccgtcgattagcgcggttcttgtcggccgcaccgagctcggcctgcagcctgatctgccggcgcacgaggcgctagacaaccacgataagcttgccgacgccctccttaaccgcgacgccgacgccgcagaaactgcgtcccgaaacatcctcaatgaggtgcgcagcgcgctgggcacgctgaactaa

SEQ ID NO: 7 - protein, 250 aa, Corynebacterium glutamicum ATCC 13032
  REGION 1..250: note = gluconate repressor protein variant GntR1_R102C wherein the aminoacid Arg in position 102 of the wildtype sequence is replaced bythe amino acid Cys
MTPANESPMTNPLGSAPTPAKPLLDSVLDELGQDIISGKVAVGDTFKLMDIGERFGISRTVAREAMRALEQLGLVASSRRIGITVLPQEEWAVFDKSIIRWCLNDEGQREGQLQSLTELRIAIEPIAARSVALHASTAELEKIRALATEMRQLGESGQGASQRFLEADVTFHELILRYCHNEMFAALIPSISAVLVGRTELGLQPDLPAHEALDNHDKLADALLNRDADAAETASRNILNEVRSALGTLN

SEQ ID NO: 8 - DNA, 1514 bp, Corynebacterium glutamicum ATCC 13032
  misc_feature 1..1514: note = polynucleotide called delta_gntR2 comprising the upstreamsequence (5-flanking sequence) and the downstream sequence(3-flanking sequence) of the coding sequence of gntR2
  source 1..1514: mol_type = other DNA
gaattcagatctagaatcactgttccagcagctctaccacacagatctacctgaaccatccatcaaagacagtggtcttatcagtgctatcggctctagcgccggcaataccaataatccagcactcgccctagaaactcagatggcttaccacctggtgcttgctatgcaccacaccgatgttgctacctggcacaaggtggtgaccaaaaacatcaccgaatctgctgctgcacaagatgctgcggtcgagcacagtgctaaatacgatgctgtgtacgatgccgcacaacttatgggcatcactgttgaggaaggtaatgtcggtagcatcgctattgcctttagcacagcacgtgcagacggtaaatctgattggtgtgtttccggcatcagccgctacatcgaggtcaccgaagccttggatgctgcgcgagctgtcactaaaaatactgctgcgctcaataaaactgctctaccagacgtgcagccggcgccggttgtgcattcagcacagttcatgaacaagtccgcacacgatcatggggttaatactgcggaaaaagatcaaccaaccctgttttaaaagactgtccatttaacaaccacatcgttacccccgaacagtcttttaaaggctattcaggggtaattttttcgccacactcccaatatctaccaaaaatggtgatctattatacataatggaattaccaaagcttcatatcacttttccacagcctgaaagaacatactttgccactaaacgagtcactacacaattacatcgctcattgttacttaattaccctttaatagtcttttacaaggctgttaaagggtaattttttattagtttgcttaaagcctattacatgacaattacagcacaattgaaaagtcacttaagcgcacgctaaaagcgaattgtagagggttatttttttcgcaattaaaagccttttgcgacacaaataggacaacaaaacaaagatgcattaactctaaaagaacaaaattaatcaatcagaaaaacatattgaatacttataaatttctgacatactcattaatgagatattcgaagtctttatcaaaatgattaacaaaaggagtatgtttatgtcgctaaaaactcgccgaatattcggcgcacttgctgtttcgctatcaatctctttctcagccattgctacacctgcagcatccgcacaagaactagtggtgagcacatcagcagtaaacgaatttggtgtagttaccagtgacatcacggctgagcaaattcttcaggcgcaagatctaatcgctgagatgaaacagtcagaggacatatatgagtatttcggtgccttgtctgacgttgaacagagatccatcattgcagctgtaaaggaaaatccatatctcattgagaacgaatcaccccgtatgagagtccaaagtgaaacacccgacgaggaaacacctgataagaaaaagccgagcaaaacctacaagctctatcctgcagg

SEQ ID NO: 9 - protein, 250 aa, Corynebacterium glutamicum ATCC 13032
  REGION 1..250: note = GntR1
MTPANESPMTNPLGSAPTPAKPLLDSVLDELGQDIISGKVAVGDTFKLMDIGERFGISRTVAREAMRALEQLGLVASSRRIGITVLPQEEWAVFDKSIIRWRLNDEGQREGQLQSLTELRIAIEPIAARSVALHASTAELEKIRALATEMRQLGESGQGASQRFLEADVTFHELILRYCHNEMFAALIPSISAVLVGRTELGLQPDLPAHEALDNHDKLADALLNRDADAAETASRNILNEVRSALGTLN

SEQ ID NO: 10 - protein, 246 aa, Corynebacterium glutamicum ATCC 13032
  REGION 1..246: note = GntR2
MSAALPHTAADPVHTTPAKPLLDHVLDSLGRSIISGEMEAGSTFKLQDIGEKFGISRTVAREAMRALEQLGLVASSRRIGITVLSHEHWAVFDKAIIRWRLEDERQREQQLQSLTELRIAIEPIAARSVALHASSAEIAIIGDLAARMRNLGEAGRGASQEFLDADVKFHELILQYCHNEMFAAMAPPIKAVLVGRTTLGLQPDRPAEEVLDNHDALAHALSVRNADLAEKASRSILNEVRDALTS

SEQ ID NO: 11 - protein, 421 aa, Corynebacterium glutamicum ATCC 13032
  REGION 1..421: note = LysC_T311I
MALVVQKYGGSSLESAERIRNVAERIVATKKAGNDVVVVCSAMGDTTDELLELAAAVNPVPPAREMDMLLTAGERISNALVAMAIESLGAEAQSFTGSQAGVLTTERHGNARIVDVTPGRVREALDEGKICIVAGFQGVNKETRDVTTLGRGGSDTTAVALAAALNADVCEIYSDVDGVYTADPRIVPNAQKLEKLSFEEMLELAAVGSKILVLRSVEYARAFNVPLRVRSSYSNDPGTLIAGSMEDIPVEEAVLTGVATDKSEAKVTVLGISDKPGEAAKVFRALADAEINIDMVLQNVSSVEDGTTDIIFTCPRSDGRRAMEILKKLQVQGNWTNVLYDDQVGKVSLVGAGMKSHPGVTAEFMEALRDVNVNIELISTSEIRISVLIREDDLDAAARALHEQFQLGGEDEAVVYAGTGR